European Patent Application EP 4 438 724 A1, published October 2, 2024. Title: 糖苷水解酶及其制备方法和应用. Applicant: 山东恒鲁生物科技有限公司. The sequence listing filed with the application follows.

SEQUENCE LISTING (2 sequences)

SEQ ID NO: 1 - protein, 722 aa, Bacillus mycoides
MKKKKGRVTLPSEENFLKETKELMERWGADAIRDSDGTKLDDDIKQLDAKIYTTYFVARAHNEFAEKHMDECQQLYLMSLFNTSLTDTLEIDFMKGYFEEQLKPDYVHNPKKYWEVIDRTTGEVVDVNDWEVNEEQNRVLITKAIPWHEYTVSFLVYAIWDPTQMYNHITNNWGDKPHDIPFDVRQPHSNEFMKTYLKQWLTENPDTDVVRFTTFFYHFTLVFNNLGKEKFVDWFGYGASVSVAALDTFQKEKGYRLRPEDIVDQGYYNTAFRIPTPAFLDYIDFVHKFVAEEAKKLVDIVHESGKEAMMFLGDNWIGTEPYGKYFENIGLDAVVGSVGGGATLRMIADIPHVRYTEGRFLPYFFPDTFYEGNNPTIEANENWLTARRALLRNPVDRIGYGGYLSLAYQFPEFISYIEKVTEEFREIHDTIKGVQPYSGLKVAILNSWGKLRTWQTHMVAHALWYKQIYSYLGVLESLSGAAVEVSFISFDDVINDGIPEDIDVIINAGDVGTAFSGGANWINEKLVTTIRAWMYNGGGFIGIGEPTAYQHEGHYFQLANVLGVDKELGFSLSTDKYFINPVENHFISADSTQFDFGEGMKNIYALSEETEIIEYSNGEVHLSSHQFGEGRSVYIAGLPYSEENTRLLMRALYYAAHKEAEFHKYHASNIYCEVHAYPSIQKMAIVNNSMIEQKTVVYDGQGNRKEVTLAPSEIRWEDVSNE

SEQ ID NO: 2 - protein, 751 aa, Bifidobacterium longum
MTSTGRFTLPSEENFAEKTKELAELWGADAIRNSDGTHLDEAVLALGKKIYSAYFPTRAHNEWITLHMDETPQVYLLTARILAESNAVDVPLMDGFFEEQLKPNRDADPHKYWEVVDRTTGEVVDPSGWTLDPGEDTVHVTAAVPMHEYTVSFLAYIIWDPVEMYNHLTNDWGDKEHEIPFDIYHPATRKFVFDTFEQWLKDSPQVDVVRFTTFFYQFTLLFDAKRREKVVDWFGCACTVSPRALDDFEKEYGYRLRPEDFVDGGAYNSAWRVPRKAQRDWIDFLSGFVRENVKRLADMSHAAGKEAMMFLGDQWIGTEPYKDGFEKLGLDAVVGSIGDGTTTRMIADIPGVKYTEGRFLPYFFPDTFYEGNDPSIEGLDNWRKARRAILRSPISRMGYGGYLSLAAKFPKFVDTVTHIANEFRDIHDRTGGVAAEGELNVAILNSWGKMRSWMAFTVAHALPNKQTYSYYGILESLSGMRVNVRFISFDDVLAHGIDSDIDVIINGGPVDTAFTGGDVWTNPKLVETVRAWVRGGGAFVGVGEPSSAPRFQAGRFFQLADVIGVDEERYQTLSVDKYFPPVVPDHFITADVPVDPAAREAWEQAGYRIPLSGCGGGQSIKPLGGIDFGEPVLNTYPVNENVTLLRADGGQVQLATNDYGKGRGVYISGLPYSAANARLLERVLFYASHNEDKYAAWSSSNPECEVAHFPEQGLYCVINNTDQPQKTTVTLADGTTEDFDLPDSGIAWREA